European Patent Specification EP 3 746 111 B1, published July 19, 2023. Title: SOLID COMPOSITIONS COMPRISING A GLP-1 AGONIST AND A SALT OF N-(8-(2-HYDROXYBENZOYL)AMINO)CAPRYLIC ACID. Applicant: Novo Nordisk A/S. The sequence listing filed with the application follows.

SEQUENCE LISTING (6 sequences)

SEQ ID NO: 1 - protein, 31 aa, Homo sapiens
HAEGTFTSDVSSYLEGQAAKEFIAWLVKGRG

SEQ ID NO: 2 - protein, 40 aa, Heloderma suspectum
HGEGTFITSDLSKQMEEEAVRLFIEWLKNGGPSSGAPPPS

SEQ ID NO: 3 - protein, 29 aa, Homo sapiens
HSQGTFTSDYSKYLDSRRAQDFVQWLMNT

SEQ ID NO: 4 - protein, 31 aa, Artificial Sequence
  Synthetic
  MOD_RES (2)..(2): Aib
  MOD_RES (20)..(20): The amino acid residue is modified with a substituent.
HXEGTFTSDVSSYLEGQAAKEFIAWLVRGRG

SEQ ID NO: 5 - protein, 31 aa, Artificial Sequence
  Synthetic
  MOD_RES (2)..(2): Aib
  MOD_RES (20)..(20): The amino acid residue is modified with a substituent.
  MOD_RES (31)..(31): The amino acid residue is modified with a substituent.
HXEGTFTSDVSSYLEGQAAKEFIAWLVRGRK

SEQ ID NO: 6 - protein, 33 aa, Artificial Sequence
  Synthetic
  MOD_RES (2)..(2): Aib
  MOD_RES (21)..(21): The amino acid residue is modified with a substituent
  MOD_RES (30)..(30): The amino acid residue is modified with a substituent
HXEGTFTSDVSSYLEEQAARKFIEWLVRGKGEG